European Patent Application EP 4 461 135 A1, published November 13, 2024. Title: COMPOSITION COMPRISING BACILLUS SIAMENSIS STRAIN FOR PROMOTING PLANT GROWTH. Applicant: Bioibérica, S.A.U. The sequence listing filed with the application follows.

SEQUENCE LISTING (4 sequences)

SEQ ID NO: 1 - DNA, 1542 bp, Bacillus siamensis
  source 1..1542: mol_type = genomic DNA
acctgcaggcggccgcactagtgattagagtttgatcatggctcaggacgaacgctggcggcgtgcctaatacatgcaagtcgagcggacagatgggagcttgctccctgatgttagcggtggacgggtgagtaacacgtgggtaacctgcctgtaagactgggataactccgggaaaccggggctaataccggatggttgtctgaaccgcatggttcagacataaaaggtggcttcggctaccacttacagatggacccgcggcgcattagctagttggtgaggtaacggctcaccaaggcgacgatgcgtagccgacctgagagggtgatcggccacactgggactgagacacggcccagactcctacgggaggcagcagtagggaatcttccgcaatggacgaaagtctgacggagcaacgccgcgtgagtgatgaaggttttcggatcgtaaagctccgttgttagggaagaacaagtgccgttcaaatagggcggcaccttgacggtacctaaccagaaagccacggctaactacgtgccagcagccgcggtaatacgtaggtggcaagcgttgtccggaattattgggcgtaaagggctcgcaggcggtttcttaagtctgatgtgaaagcccccggctcaaccggggagggtcattggaaactggggaacttgagtgcagaagaggagagtggaattccacgtgtagcggtgaaatgcgtagagatgtggaggaacaccagtggcgaaggcgactctctggtctgtaactgacgctgaggagcgaaagcgtggggagcgaacaggattagataccctggtagtccacgccgtaaacgatgagtgctaagtgttagggggtttcctccccttagtgctgcagctaacgcattaagcactccgcctggggagtacggtcgcaagactgaaactcaaaggaattgacgggggcccgcacaagcggtggagcatgtggtttaattcgaagcaacgcgaagaaccttaccaggtcttgacatcctctgacaatcctagagataggacgtccccttcgggggcagagtgacaggtggtgcatggttgtcgtcagctcgtgtcgtgagatgttgggttaagtcccgcaacgagcgcaacccttgatcttagttgccagcattcagttgggcactctaaggtgactgccggtgacaaaccggaggaaggtggggatgacgtcaaatcatcatgccccttatgacctgggctacacacgtgctacaatgggcagaacaaagggcagcgaaaccgcgaggttaagccaatcccacaaatctgttctcagttcggatcgcggtctgcaactcgactgcgtgaagctggaatcgctagtaatcgcggatcagcatgccgcggtgaatacgttcccgggccttgtacacaccgcccgtcacaccacgagagtttgtaacacccgaagtcggtgaggtaaccttttaggagccagccgccgaaggtgggacagatgattggggtgaagtcctaacaaggtaaccgaatc

SEQ ID NO: 2 - protein, 6 aa, synthetic construct
  source 1..6: note = circular
  REGION 1..6: note = circular
GLVIAF

SEQ ID NO: 3 - DNA, 20 bp, synthetic construct
  source 1..20: mol_type = other DNA
agagtttgatcatggctcag

SEQ ID NO: 4 - DNA, 24 bp, synthetic construct
  source 1..24: mol_type = other DNA
cggttaccttgttaggacttcacc